European Patent Specification EP 3 822 353 B1, published August 27, 2025. Title: METHOD FOR THE PRODUCTION OF dsRNA. Applicant: CONSEJO SUPERIOR DE INVESTIGACIONES CIENTÍFICAS (CSIC) UNIVERSITAT POLITÈCNICA DE VALÈNCIA. The sequence listing filed with the application follows.

SEQUENCE LISTING (24 sequences)

SEQ ID NO: 1 - DNA, 100 bp, Ceratitis capitata
gctgaccgaagcaccgttgaacccgaaggctaaccgcgagaagatgacccagatcatgttcgagaccttcaactcgccggccatgtatgtggccatccag

SEQ ID NO: 2 - DNA, 100 bp, Ceratitis capitata
ctggatggccacatacatggccggcgagttgaaggtctcgaacatgatctgggtcatcttctcgcggttagccttcgggttcaacggtgcttcggtcagc

SEQ ID NO: 3 - DNA, 413 bp, Tetrahymena thermophila
aaatagcaatatttacctttggagggaaaagttatcaggcatgcacctggtagctagtctttaaaccaatagattgcatcggtttaaaaggcaagaccgtcaaattgcgggaaaggggtcaacagccgttcagtaccaagtctcaggggaaactttgagatggccttgcaaagggtatggtaataagctgacggacatggtcctaaccacgcagccaagtcctaagtcaacagatcttctgttgatatggatgcagttcacagactaaatgtcggtcggggaagatgtattcttctcataagatatagtcggacctctccttaatgggagctagcggatgaagtgatgcaacactggagccgctgggaactaatttgtatgcgaaagtatattgattagttttggagtactcg

SEQ ID NO: 4 - DNA, 10 bp, Tetrahymena thermophila
atgactctct

SEQ ID NO: 5 - DNA, 10 bp, Tetrahymena thermophila
taaggtagcc

SEQ ID NO: 6 - DNA, 433 bp, Artificial Sequence
  Autocatalytic intron flanked by exon fragments
atgactctctaaatagcaatatttacctttggagggaaaagttatcaggcatgcacctggtagctagtctttaaaccaatagattgcatcggtttaaaaggcaagaccgtcaaattgcgggaaaggggtcaacagccgttcagtaccaagtctcaggggaaactttgagatggccttgcaaagggtatggtaataagctgacggacatggtcctaaccacgcagccaagtcctaagtcaacagatcttctgttgatatggatgcagttcacagactaaatgtcggtcggggaagatgtattcttctcataagatatagtcggacctctccttaatgggagctagcggatgaagtgatgcaacactggagccgctgggaactaatttgtatgcgaaagtatattgattagttttggagtactcgtaaggtagcc

SEQ ID NO: 7 - DNA, 333 bp, Eggplant latent viroid
gggtggtgtgtgccacccctgatgagaccgaaaggtcgaaatggggtttcgccatgggtcgggactttaaattcggaggattcgtcctttaaacgttcctccaagagtcccttccccaaacccttactttgtaagtgtggttcggcgaatgtaccgtttcgtcctttcggactcatcagggaaagtacacactttccgacggtgggttcgtcgacacctctccccctcccaggtactatcccctttcaaggatgtgttccctaggagggtgggtgtacctcttttggattgctccggccttccaggagagatagaggacgacctctccccata

SEQ ID NO: 8 - DNA, 247 bp, Avocado sunblotch viroid
tttattagaacaagaagtgaggatatgattaaactttgtttgacgaaaccaggtctgttccgactttccgactctgagtttcgacttgtgagagaaggaggagtcgtggtgaacttttattaaaaaaattagttcactcgtcttcaatctcttgatcacttcgtctcttcagggaaagatgggaagaacactgatgagtctcgcaaggtttactcctctatcttcattgtttttttacaaaatcttg

SEQ ID NO: 9 - DNA, 399 bp, Chrysanthemum chlorotic mottle viroid
ggcacctgacgtcggtgtcctgatgaagatccatgacaggatcgaaacctcttccagtttcggcttgtgtgggagtaaagctttcgctctctccacagcctcatcaggaaacccacttcaggtctcgactggaaggtcgttaaacttcccctctaagcggagtagaggtaaatacctccgtccaaccccgggaggaaaggggttgggacccggaacagatccagttccggtcctttggagtccatttctctcgttggatattctcctcggagaagggagatggggccagtcccagtcggttcgctctcgtagtcacagccactggggaacctaggcagatggctggacggagtcttagtccactccagaggaccttgggtttgaaacccccaagaggtc

SEQ ID NO: 10 - DNA, 337 bp, Peach latent mosaic viroid
gtcataagtttcgtcgcatttcagcgactcatcagtgggcttagcccagacttatgagagagtaaagacctctcagcccctccaccttggggtgccctattcggagcactgcagttcccgatagaaaggctaagcacctcgcaatgaggtaaggtgggacttttccttctggaaccaagcggttggttccgaggggggtgtgatccaggtaccgccgtagaaactggattacgacgtctacccgggattcaaacccgtcccctccagaagtgattctggatgaagagtctgtgctaagcacactgacgagtctctgagatgagacgaaactcttctt

SEQ ID NO: 11 - DNA, 386 bp, Eggplant latent viroid
ccccatagggtggtgtgtgccacccctgatgagaccgaaaggtcgaaatggggtttcgccatgggtcgggactttaaattcggaggattcgtcctttaaacgttcctccaagagtcccttccccaaacccttactttgtaagtgtggttcggcgaatgtaccgtttcgtcctttcggactcatcagggaaagtacacactttccgacggtgggttcgtcgacacctctccccctcccaggtactatcccctttcaaggatgtgttccctaggagggtgggtgtacctcttttggattgctccggccttccaggagagatagaggacgacctctccccatagggtggtgtgtgccacccctgatgagaccgaaaggtcgaaatgggg

SEQ ID NO: 12 - DNA, 1019 bp, Artificial Sequence
  A plant viroid comprising the cDNAs of two strands of a target dsRNA Separated by an autocatalytic intron flanked by exon fragments inserted in its nucleotide sequence.
ccccatagggtggtgtgtgccacccctgatgagaccgaaaggtcgaaatggggtttcgccatgggtcgggactttaaattcggaggattcgtcctttaaacgttcctccaagagtcccttccccaaacccttactttgtaagtgtggttcggcgaatgtaccgtttcgtcctttcggactcatcagggaaagtacacactttccgacggtgggttcgtcgacacctctccccctcccaggtactatccccttgctgaccgaagcaccgttgaacccgaaggctaaccgcgagaagatgacccagatcatgttcgagaccttcaactcgccggccatgtatgtggccatccagatgactctctaaatagcaatatttacctttggagggaaaagttatcaggcatgcacctggtagctagtctttaaaccaatagattgcatcggtttaaaaggcaagaccgtcaaattgcgggaaaggggtcaacagccgttcagtaccaagtctcaggggaaactttgagatggccttgcaaagggtatggtaataagctgacggacatggtcctaaccacgcagccaagtcctaagtcaacagatcttctgttgatatggatgcagttcacagactaaatgtcggtcggggaagatgtattcttctcataagatatagtcggacctctccttaatgggagctagcggatgaagtgatgcaacactggagccgctgggaactaatttgtatgcgaaagtatattgattagttttggagtactcgtaaggtagccctggatggccacatacatggccggcgagttgaaggtctcgaacatgatctgggtcatcttctcgcggttagccttcgggttcaacggtgcttcggtcagctcaaggatgtgttccctaggagggtgggtgtacctcttttggattgctccggccttccaggagagatagaggacgacctctccccatagggtggtgtgtgccacccctgatgagaccgaaaggtcgaaatgggg

SEQ ID NO: 13 - protein, 1167 aa, Solanum melongena
MSVSHRVIYSFTHYKLYNLSSSLSSLPSRIFFPFQSPSFHTFSSLMPNNQERGGYEGKKWQVRPSSNRVPGSSSNVEPVSAATAEAITDRLKSVDITESGAQSSVPVTSLQFGSVGLAPQSPVQHQKVIWKPKSYGTVSGAPVVEAGKTPVEQKSALLSKLFKGNLLENFTVDNSTFSRAQVRATFYPKFENEKSDQEIRTRMIEMVSKGLAIVEVTLKHSGSLFMYAGHEGGAYAKNSFGNIYTAVGVFVLGRMFREAWGTKASKKQAEFNEFLERNRMCISMELVTAVLGDHGQRPRDDYAVVTAVTELGNGKPTFYSTPDVIAFCREWRLPTNHVWLFSTRKSVTSFFAAYDALCEEGTATTVCEALSEVADISVPGSKDHIKVQGEILEGLVARIVKRESSEHMERVLRDFPPPPSEGEGLDLGPTLREICAANRSEKQQIKALLQSAGTAFCPNYLDWFGDENSGSHSRNADRSVVSKFLQSHPADLYTGKIQEMVRLMREKRFPAAFKCHYNLHKINDVSSNNLPFKMVIHVYSDSGFRRYQKEMRHKPGLWPLYRGFFVDLDLFKVNEKKTAEMAGSNNQMVKNVEEDNSLADEDANLMVKMKFLTYKLRTFLIRNGLSTLFKEGPSAYKSYYLRQMKIWNTSAAKQRELSKMLDEWAVYIRRKYGNKPLSSSTYLSEAEPFLEQYAKRSPQNHALIGSAGNFVKVEDFMAIVEGEDEEGDLEPAKDIAPSSPSISTRDMVAKNEGLIIFFPGIPGCAKSALCKEILNAPGGLGDDRPVNSLMGDLIKGRYWQKVADERRRKPYSIMLADKNAPNEEVWKQIENMCLSTGASAIPVIPDSEGTETNPFSIDALAVFIFRVLHRVNHPGNLDKSSPNAGYVMLMFYHLYDGKSRQEFESELIERFGSLVRIPVLKPERSPLPDSVRSIIEEGLSLYRLHTTKHGRLESTKGTYVQEWVKWEKQLRDILLGNADYLNSIQVPFEFAVKEVLEQLKVIARGEYAVPAEKRKLGSIVFAAISLPVPEILGLLNDLAKKDPKVGDFIKDKSMESSIQKAHLTLAHKRSHGVTAVANYGSFLHQKVPVDVAALLFSDKLAALEAEPGSVEGEKINSKNSWPHITLWSGAGVAAKDANTLPQLLSQGKATRIDINPPVTITGTLEFF

SEQ ID NO: 14 - DNA, 3848 bp, Solanum melongena
gtgactggctcaaaggcggtagtagtggctcttcttccccgctggaatttctcgcctattttatattgattgacagcagccgagtcttccttttgtgtagaactgaatgtcggtttcgcatagggtcatttactctttcactcattacaaactctataatctctcttcttctttatcatctttgccttctagaatcttcttcccttttcaatctccttcctttcacacgttctcttcactcatgcccaacaatcaggaaaggggtggttatgaaggaaaaaaatggcaagtgaggccaagttccaatagggtaccaggctcgtcttcaaatgtggaacctgtatctgctgcaactgctgaagccattaccgaccgtctaaagtccgtggatattactgaaagtggtgcacagtctagtgttccagtcacatctcttcagtttggcagcgttggattagcaccccagtcacctgtgcaacatcaaaaagtaatctggaaacccaaatcatatggaacagtgtctggagccccagtggttgaagctggaaaaacaccagttgaacaaaaaagtgctcttttaagtaaattattcaagggtaatttattggaaaattttactgtagataactcaacattctcgagagcccaagtaagggccactttctacccaaaatttgagaatgagaaatcagatcaggagatcaggacaaggatgatagagatggtctccaaaggcttggctatagtcgaggtcacacttaagcattctggatctctttttatgtatgctgggcatgaaggtggagcatatgccaagaatagcttcgggaatatctatactgccgttggcgtctttgttcttggacggatgtttcgtgaggcatggggaactaaagcaagcaagaagcaagcagagttcaatgagtttcttgagcgcaatcgtatgtgcatatcaatggagttggtcacggcagtgttgggggaccacggacaacgcccacgagatgattatgcggttgtgactgcagtcacggagttgggaaatggaaaaccaactttctattcaactcccgatgtaattgctttttgcagggaatggcgattaccaacaaatcatgtatggctgttctcaacaaggaaatcagtgacttccttctttgctgcgtatgatgcactttgcgaggaaggtacagcaaccaccgtttgcgaggctctcagcgaagttgctgatatttctgtacctggatcaaaagaccatataaaagtgcagggtgaaattttggagggtctcgtggcccgcatcgtaaaacgtgagagctcagagcatatggagcgggttctgagagattttcctcctccgccatcagagggtgagggtttggacctgggacctacgttacgtgaaatttgtgctgcaaacagatcagaaaagcagcaaataaaggcacttcttcagagtgctggcacggctttctgcccgaattatttggactggtttggagatgaaaactctggttcacattcaagaaatgctgatcgatctgttgtctcaaagttcttacaatcacatcctgctgatctttatacaggaaaaatacaggaaatggttcgcttgatgagggaaaagcgctttcctgctgctttcaagtgtcattataacttacataaaattaatgatgtatcgagtaacaacctgcctttcaaaatggtgatccatgtatatagtgattcaggcttccgccggtaccagaaagagatgaggcacaaaccaggactatggcctttgtatcgaggcttttttgttgacctggatttattcaaggtcaatgagaagaaaactgctgaaatggcaggaagcaacaatcaaatggtaaaaaatgtggaagaggacaacagtttagctgatgaagatgcaaatctgatggtcaagatgaaatttcttacttacaagttgagaacttttttgatccgtaatggcttgtcgactcttttcaaagaaggaccttctgcgtataagtcttattacctgaggcaaatgaaaatttggaatacttcagcagccaagcaacgagaactcagcaagatgcttgatgaatgggcagtatatatacgcagaaaatatgggaacaaaccattgtcatcatccacatacctaagtgaagctgagcctttccttgaacaatatgcaaagcgtagtccacaaaatcatgctttgataggatctgctggaaattttgtcaaagttgaagatttcatggctattgttgaaggagaagatgaagagggtgatctcgagcctgcgaaagatattgctccttcaagccctagtatttccaccagagacatggtggcaaagaatgagggtctcattattttctttccaggaataccaggttgtgctaaatctgcactttgtaaggaaatactgaatgctccaggagggcttggagatgatcgaccagttaacagtttaatgggtgatcttattaaaggtagatattggcaaaaagttgctgatgaacgtcgaagaaaaccttactcgatcatgcttgctgacaagaatgcaccaaatgaggaagtatggaaacaaattgagaacatgtgcctaagcaccggagcatctgctattccagttatacctgattcagaaggaactgaaactaatccattctctattgatgcacttgcggtttttatattccgagtacttcaccgtgtcaatcatccgggaaatcttgacaagtcatctccaaatgctggatatgtgatgcttatgttttatcacctttatgatggaaagagccgtcaggagttcgagagtgagcttattgaacgttttggatcgcttgtcagaattcctgtactgaaacctgagaggtctcctcttccggattctgtgaggtctattatcgaggagggactcagtctgtacagacttcatacaacgaaacatggaagattggagtctacaaaagggacatatgtacaagagtgggttaaatgggagaagcaattgagagatattctacttggaaatgcagactatctcaattcaatacaggttccatttgaatttgccgttaaagaagtccttgaacaactgaaagttattgcgaggggcgaatatgcagtgcctgctgagaagaggaagctaggatccattgtattcgccgctatcagcctgccagttccagaaattctaggtcttctaaatgatctagcaaagaaagatccaaaggttggcgatttcattaaggacaagagcatggagagcagcattcagaaggcccatcttaccctggctcacaagagaagtcacggtgtcactgcagttgccaattacggttcctttcttcatcaaaaggtgccagtagacgtggctgctttgttgttctccgataaattggctgcactagaagctgagcctggctctgttgaaggtgaaaagatcaattctaaaaactcatggccccatatcacattatggtctggtgcaggagttgccgcaaaagatgccaatacactaccacagttactttcccaagggaaggctacccgcattgatataaatccaccggtcactataactggcactctcgaattcttttgaactctacttgtaattcctcttgtgtggatttacataatgtgaaccctacatgggttctgagtgaatcatgtaatgattctcctgagttttaggaacaattttgtagcagtcttgcagttgcaggatagaactagatctagagaaaatgtaaagatgtttaaggcaataaaggtcttgagctgtgggcatattgaaaatccccagtagcatttttcttgagcaaaaaaaaaaaaaaaaa

SEQ ID NO: 15 - DNA, 188 bp, Tetrahymena thermophila
cttctgttgatatggatgcagttcacagactaaatgtcggtcggggaagatgtattcttctcataagatatagtcggacctctccttaatgggagctagcggatgaagtgatgcaacactggagccgctgggaactaatttgtatgcgaaagtatattgattagttttggagtactcgtaaggtagcc

SEQ ID NO: 16 - DNA, 245 bp, Tetrahymena thermophila
atgactctctaaatagcaatatttacctttggagggaaaagttatcaggcatgcacctggtagctagtctttaaaccaatagattgcatcggtttaaaaggcaagaccgtcaaattgcgggaaaggggtcaacagccgttcagtaccaagtctcaggggaaactttgagatggccttgcaaagggtatggtaataagctgacggacatggtcctaaccacgcagccaagtcctaagtcaacagat

SEQ ID NO: 17 - DNA, 1452 bp, Artificial Sequence
  Nuccleotide sequence of the invention
ccccatagggtggtgtgtgccacccctgatgagaccgaaaggtcgaaatggggtttcgccatgggtcgggactttaaattcggaggattcgtcctttaaacgttcctccaagagtcccttccccaaacccttactttgtaagtgtggttcggcgaatgtaccgtttcgtcctttcggactcatcagggaaagtacacactttccgacggtgggttcgtcgacacctctccccctcccaggtactatccccttcttctgttgatatggatgcagttcacagactaaatgtcggtcggggaagatgtattcttctcataagatatagtcggacctctccttaatgggagctagcggatgaagtgatgcaacactggagccgctgggaactaatttgtatgcgaaagtatattgattagttttggagtactcgtaaggtagccgctgaccgaagcaccgttgaacccgaaggctaaccgcgagaagatgacccagatcatgttcgagaccttcaactcgccggccatgtatgtggccatccagatgactctctaaatagcaatatttacctttggagggaaaagttatcaggcatgcacctggtagctagtctttaaaccaatagattgcatcggtttaaaaggcaagaccgtcaaattgcgggaaaggggtcaacagccgttcagtaccaagtctcaggggaaactttgagatggccttgcaaagggtatggtaataagctgacggacatggtcctaaccacgcagccaagtcctaagtcaacagatcttctgttgatatggatgcagttcacagactaaatgtcggtcggggaagatgtattcttctcataagatatagtcggacctctccttaatgggagctagcggatgaagtgatgcaacactggagccgctgggaactaatttgtatgcgaaagtatattgattagttttggagtactcgtaaggtagccctggatggccacatacatggccggcgagttgaaggtctcgaacatgatctgggtcatcttctcgcggttagccttcgggttcaacggtgcttcggtcagcatgactctctaaatagcaatatttacctttggagggaaaagttatcaggcatgcacctggtagctagtctttaaaccaatagattgcatcggtttaaaaggcaagaccgtcaaattgcgggaaaggggtcaacagccgttcagtaccaagtctcaggggaaactttgagatggccttgcaaagggtatggtaataagctgacggacatggtcctaaccacgcagccaagtcctaagtcaacagattcaaggatgtgttccctaggagggtgggtgtacctcttttggattgctccggccttccaggagagatagaggacgacctctccccatagggtggtgtgtgccacccctgatgagaccgaaaggtcgaaatgggg

SEQ ID NO: 18 - DNA, 3820 bp, Arabidopsis thaliana
agaaacgacgttgtgttcaagttactaaatcgcgtgtgttttttacttttctgcaactaaatcgtgtttcttcctaagaaccctaaatctgaactgtctcatcttctccgatatcagtgagatcaataaatcatcttctcaccctagacgacagggaaactcggggattgattcggaaaaacgagttcgtttttctgcaagaaaaagagagatcacgctgagcagaagtggcaagtaaaaccgaagatggatgctccatttgaatccggtgatagttcggcaacagttgttgcagaagcagtaaacaaccaatttggcgggttaagtcttaaggaaagcaacactaatgcgccagtcttaccgagtcaaactacaagtaaccaccgtgttcaaaatctagtatggaaacctaagtcatatggaacagttagtggatcatcttcggcaacagaagttggtaaaacatcggctgtctcacagataggttcttctggagatacaaaagttggtctcaatctgagcaaaattttcggaggtaatttgttggaaaaattttcggtggacaaatcgacttattgtcatgctcagatcagagccactttctatccaaaatttgagaacgaaaagactgaccaagagataagaacaagaatgattgagatggtatctaaaggattggcaacactggaggtatctcttaagcattcaggctctctctttatgtacgccggtcacaaggggggagcatatgcaaagaacagttttggtaatatttatactgcggttggtgtttttgttctttcacggatgttcagggaggcttggggaactaaggctccaaagaaagaagcagagttcaatgattttcttgagaaaaatcgcatgtgcatatctatggaactggtaaccgctgttcttggagatcatggtcaacgcccactggatgattatgtggtagtgactgctgttaccgagttaggtaatgggaagccccagttctattcaacttccgaaataatttcattttgccggaaatggcgtctacccacaaatcatgtttggctgttttccacaaggaaatcagtgacctcttttttcgcggcgtttgatgcactgtgtgaagaagggatagcaacctcggtctgtagagctcttgatgaagtagctgatatatcagtcccagcctcaaaggaccatgttaaggtgcagggtgagatattagagggtcttgttgctcgtatcgtgagcagtcagagctcaagagatatggaaaatgtcttgagagatcatcctccaccaccctgtgatggagctaatcttgatctgggactcagtctaagagagatatgtgctgcccatagatctaacgagaaacagcaaatgagagcacttttaaggagtgttgggccaagcttttgccccagtgacgtggaatggttcggagatgaatctcatccgaaaagtgctgacaaatctgttataacaaaattcctgcaatctcagcctgcagattattcaactagtaaattacaggaaatggtacgcttgatgaaggaaaaacgtcttccagccgcattcaagtgttaccataattttcatagagctgaggacatatcacctgataaccttttttataaattggttgtccatgtgcacagcgattcaggatttaggcgttaccacaaagagatgaggcacatgcctagtttgtggcctttatatcgaggtttctttgttgatattaatttgttcaagtcaaacaaagggagggatctgatggctctgaaaagcattgataatgccagtgaaaatgatggtcgaggagaaaaggatggtttggctgatgatgatgctaacttaatgattaaaatgaagtttctcacatacaagttgagaacctttttgatccgtaatggcctatcaattctatttaaagacggggcagcagcttacaaaacttactaccttaggcaaatgaaaatctggggtacgtcagatggaaagcagaaagaactttgcaagatgcttgatgaatgggctgcttacataagaagaaagtgtgggaatgatcagctatcttcatcaacatacttaagtgaagctgagccattcctggagcagtacgcgaaacggagcccaaagaaccatattttgatagggtctgctgggaacctagttagaactgaggacttcttggccattgttgacggtgatctagatgaagaaggcgatcttgtgaagaaacaaggagtgacaccagctactcctgagccagctgtgaaggaagctgtccaaaaggatgaggggttaattgtattctttccaggaattcctggatctgctaaatctgcactttgcaaggagttattgaacgccccaggaggctttggagatgataggccagtgcatactctgatgggtgatcttgtcaaaggaaaatattggccaaaggttgctgatgaacgtcgtaaaaaaccacaatcgattatgttggctgacaaaaatgccccaaatgaagatgtctggagacagattgaagatatgtgtcggagaactagggcttctgcagttccaatcgttgctgattctgaaggaaccgatacaaatccatattcacttgatgccttggctgtattcatgttccgtgtacttcaacgagttaaccatccgggaaagctcgacaaggaatcttcaaatgcaggttatgtgctattgatgttttatcacctttatgagggaaagaaccgtaatgaatttgagagtgaattgattgagcgctttggctccctcatcaagatgccactattgaaatcagacaggactcctttacctgatcctgttaaatcagttcttgaggagggcattgatttgttcaatctccatagtagaagacatgggagactcgagtcaacaaaaggaacatatgcagcggaatggaccaaatgggagaaacaactacgagatactctagttgcaaattctgagtatctcagttctattcaggttccatttgagtctatggttcatcaagtgcgagaagagctaaaaacaatagcgaagggtgattacaagccaccaagttcggagaaaagaaaacacgggtctattgttttcgctgccatcaacttgcctgctactcaagttcacagtcttcttgaaaagttggctgcagcaaacccaacaatgagatcttttctagagggaaagaaaaagagcatacaggaaaaacttgaacggtctcacgtgacgctcgcccacaagagaagccatggcgtagcaactgtagccagctatagtcagcacttgaacagagaggtacccgtagagctcaccgagctcatctacaacgacaagatggctgctctaacagcccatgttggatctgtggacggagagaccgtagtctccaagaacgaatggccacatgttacattgtggacagcggaaggcgttactgcgaaagaggccaacacgttacctcagctttacttagaaggaaaggcgagccgcttggtgatagatcctccggtgtcaatctcaggtcctctggagtttttctgaatacttgattaaacatggaagtttctctcttgagggaggttgctcgtggaatgggacacatatggttgttataataaaccatttccattgtcatgagattttgaggttaatatatactttacttgttcattattttatttggtgtttgaataaatgatataaatggctcttgataatctgcattcattgagatatcaaatatttactctagagaagagtgtcatatagattgatggtccacaatcaatgaaatttttgg

SEQ ID NO: 19 - DNA, 3876 bp, Solanum lycopersicum
tatggaacccaattggagagtgccggttccccctgaaattttctggcttcatctgtatacaacagttgagtcttccttttctatagcactgaatgtcggttttcgttcactctttcactgctaaactccatctccctcacaatctctcttcttcttcttcctcatatttcccttctagaatcttctttcgctttcaatctcgttccctcacacacagtacctcgctattctcttcactcatgccaaacaatcagagaaagggtggttataaagaaaaaaaatggcaagtgaggagttccaatagggtaccaggttcatcttcaaatgtcgaacctgcatctcctgcaactactggagccattgctgaccgtctaagttccttgaatattactgaaagtggtgcacagtctagtgttccagttgcatctcttcagtttggcagcgttggattagcaccccaatcacctgtgcagcatcaaaaagtcatctggaaacccaagtcatatggaacagtgtctggagccccaaagattgaagctgtaaaaacaccaaatgaacaaaaaagtgctcttttgagcaaattatttaagggtagtttattggaaaattttactgtagataactccacattctcaaaagcccaaataagggccactttctacccaaaatttgagaatgagaaatcagatcaggagattaggacaaggatgatagagatggtctccaaaggcttggctacagtggaggtctctcttaagcattctggatctctttttatgtatgctgggcataagggtggagcatatgccaagaatagctttggaaatatctatactgccgttggtgtctttgttcttggacggatgtttcgtgagacatggggtactcaagcaagtaagaagcaagcagagttcaatgagtttcttgagcgcaatcgcatgtgtatatcaatggagttggtcacggcagtgttgggggaccacggacaacgcccacgagatgattatgcggttgtgactgcagtcacggagttgggaagtggaaaaccaaatttctattcaactcccgatgtaattgctttttgcagagaatggagattaccaacaaatcatatatggctgttctcaacaaggaaatcagttacttccttctttgctgcgtttgatgcactctgtgaggaaggtacagcaacctctgtttgccaggctcttgctgaagttgctgacatttctgtacctggatcaaaagaccatataaaagtgcagggtgaaattttggagggcctcgtggcacgcattgtaaaacgtgagagctcagagcatatggagcgggttctaagagattttcctcctcctccattagagggtgagggtttggacttgggacctacgctgcgtgaggtttgtgctgcaaatagatcagaaaagcagcaaatcaaggcgcttcttcagagtgctggcacggctttctgcccgaattatttggactggtttggagatgatgattctggctcacattcaagaaatgctgatcgctctgttgtgtcaaagttcttacagtcacatcctgctgatttttctacaggaaaattacaggaaatggttcgtttgatgagggaaaaacgctttcctgctgctttcaagtgttactataacttccataaaattaatgatttatcgagtgacaacctgcctttcaaaatggtgatccacgtacatagtgattcaggcttccgccggtaccagaaagagatgagacacaaaccaggactgtggcctttgtatcgaggcttttttgttgacctggatttattcaaggtcaatgagaagaaaactgccgaaatggtaggaagtagcaatcaaatggtaaaaaatgaggaagaggatagccgtttagctgatgaagatgcaaatttgatggtcaagatgaaattccttccttacaagttgagaacttttttgatccgtaatggcttgtcgactcttttcaaagaaggcccttctgcgtataaggcttattacctgaggcaaatgaaaatatggaatacttcagcagccaagcaacgagaactcagcaagatgcttgatgaatgggcagtatatatacgcagaaaatatgggaacaaaccattgtcatcatccacatacctaagtgaagctgagcccttccttgagcaatatgcaaagtgtagtccacaaaatcaggcgttgataggatctgctggaaattttgtcaaagttgaagacttcatggctattgttgaaggagaagatgtagagggtgatcttgagccgaccaaagatattgctccttcaagccctaatatttccagcaaagacatggtcgcaaagaatgagggtctcatcgttttttttccaggaataccaggttgtgctaaatctgcactttgtaaggaaatactgaatgctccaggagggcttgaagatgatcggccaattcatagtttaatgggtgatcttatcaaaggtagatattggcaaaaagttgctgatgaacgtcgaagaaaaccttactcgatcatgcttgctgacaagaatgcaccaaatgaggaagtatggaaacaaattgagaacatgtgtctaagcaccaaagcatctgctattccagttatacctgattcagaaggaactgaaatcaatccattctctattgatgcactggcggtttttatattccgagtacttcagcgtgttaatcatccgggaaatcttgacaagtcatctccaaatgctggatatgtgatgttaatgttttatcacctttatgatggaaagagccgtcaggagttcgagagtgaacttattgaacgttttggatcacttgtcagaattcctctactgaaacctgaaaggtctcctcttccggattctgtgaggtctattgttgaggagggaatcaatctgtacaggcttcatactaacaaacatggaagattggagtctacaaaagggacttttgtaaaagagtgggttaaatgggagaagcaattgagggatattctacatggaaatgcggactatctcaattcaatacaggttccatttgaatttgctgttaaaaaagtccttgaacaactgaaagctattgcgaggggcgaatatgcagctccttcttctgagaagaggaagctaggatccattgtgtttgccgctatcagcctgccagttccagaaattctaggtcttctgaatgatctagccaagaaagatctgaaggttggtgatttcttgaaggacaaaagcctggagagctgcattcagaaagcccatttgaccctagctcacaagagaagtcatggtgtcactgcagttgccaattacggttcctttcttcaccaaaacgtcccagtagacgtggctgctttgttgttctccgataaattggctgccctagaagctgagcctggttctgtcgaaggtgaaaaggtcgattctaaaaacccatggccccacgtcacaatatggactggggcaggagctacagccaaagatgccaatacactaccacagttactttctcaagggaaggctatccgcattgatattaatccacccgtcactataactggcactctcgaattcttttgaactctacatgtaattcctcatcttgtgtggatttacctaatgtaaaccctacatgggttctgagtgaatatcatgtaatgacactcccgagttgtaggaacaattttgtaggatcgtgcgctttggctatatagcagtcttgcagttgcaggatagaaatagatttagagaaaatgtaaagatgttgaggcaataaaggtcttaagtcgtgggcgttttgaaatccccgatggcatttcttgaataaagcacaccattttctaccctt

SEQ ID NO: 20 - DNA, 3860 bp, Hevea brasiliensis
gcctgctaactccttctcccctttttttctcctactggcagttagtagagacattgaaccccaaaacctctccagaaacctccacctgcaactttttgcgctactgagtcacccactctctctctctccctctctctctctctctccctctctctccgttctttcggttactatttatagccattgccacaccaactatgcgaagcatcctcttcacactttctctgactctcccgttttctcctccttccctaaacctcaaatctaaaagcttcattttccttcgatcttctccttcctttttagccctacctcgctcttcttctctttccatttctcatctaatcatgtctcagagaaagggcgggcttgaaggacaacagtggaaaccgaatccaaccacggaccagccgtctccctccggtctgggtgcatcggttgcggcggttaccgatagaattggtggtttgagtatagccgaaagcagtggccagagtcatgttgtggagccattgcccgtgccgtttggtaatgcgcaagtggttaatcagtgtaacttgcaaggtcaaaaggctatatggaagcctatgtcctatggaacagtaagtggagcttcaactgtggaagttgaaaatgtgccttctaatggaatgctggttgatgtccagagcagtgcgtctggtacagcttcggtggcagctcggaagagtagtgttaacttgagtcaattctttaggggtaatctgttagaaaattttgctgtggataattcgacttattcacaagcccaaattagagccactttctatcccaaatttgaaaatgagaagtctgatcaggagattaggatcagaatgatagagatggtatctaaagggctggctacattggaggtcacactcaagcattctgggtctctttttatgtatgcgggtcataagggtggagcatatgcaaaaaatagcttcggaaatatatacactgctgttggtgtctttgttcttggtcgaatgtttcatgaggcatggggaaccgcagctgcaaaaaagcaagcagagttcaatgagtttcttgagagaaaccgaatgtgtatatcaatggaattggtaactgcagttctaggagaccatgggcaacgaccccgagaggattatgtggtggtcacagcagtcacagagttaggcaatggaaagccaaagttctactcaactcctgaattgattgccttttgtcgaaaatggcgccttccaacaaatcatgtttggctgttctcaacgaggaaatcagtaacgtctttttttgctgcctatgatgcactatgtgaagaaggaacagcaaccactgtatgtagggctcttgatgaagttgctgatatttctgtcccaggttcaaaagaccatataaaggtgcagggtgaaatcctggagggtcttgttgctcggattgtaggtcctgacagctcaaaacacatggaggatgtcttgagggaacatcctccttcaccagctgaaagagcggaccttgatttgggactaagtctaagagaaatttgtgctgctaatagggctgatgaaaaacagcaaataaaagcgctacttcagagcattggctcttctttttgccctgacaattcagactggtttgggattgaaggtggtgatacccattcaagaaatgctgacagatctgttgtttcaaaatttttacaagctcaccccactgattattcaaccaagaagttgcaggaaatggttcgtttgctgagagaaagacgcttcccagctgcttttaaatgttaccataacttccaaaaaattgattctgtatcaagtgacaaccttttctacaagatggttattcatgtccacagtgactctggatttcggcgatatcaaaaagagatgaggcacaagccagggttgtggccattgtatcgaggtttttttgttgacatcaatttattcaaggcaaacaaggagagagctgctgaaattgcaaaaaataacaataacatggaggaaactattaatggcaatgatgctgtatctgcaaaagatggtatagctgacgaagatgcaaatttaatgataaaattaaaatttcttacatataagttaagaacctttttgatccgcaatggtttgtcgattcttttcaaggatggtccatctgcttacaaggcctactacctgaggcagatgaaaatatggggcacatcagctggaaagcagagagaactcagcaagatgcttgatgaatgggctgtctacatccgaagaaaacatggaaagaaacagttgtcatcctcaatataccttagtgaagctgagccttttcttgaacagtatgcaagtcgaagtccagagaatcaggctctgataggatctgctggaagtttagttagggctgaagatttcttggccattataggagacagggatgaagagggtgatcttgagacagagcgagaggtggcgcccccgagccctatgtcctcagtcaaggacactgttcaaaagaatgagggtttaattgtattttttccaggaatacctggttgtgctaagtctgctctttgcaaggaattactaaatgcccctggaggacttggagatgatcgccctgtccatagtttgatgggggaccttatcaaaggaaagtattggcagaaggttgctgaggagcgcaggagaaaaccatattctataatgctggctgacaagaatgcaccaaatgaagaagtttggagacagattgaagatatgtgccgtagcacccgagcgtcagctgttcctgttatacctgattctgaaggaacagattcaaatccattttctcttgatgcattatcagttttcattttccgtgttcttcaacgagttaatcatccgggaaatctggacaaagcatctccaaatgctggttacgtgcttttaatgttttatcatctttatgatggcaagagtcaacaagagtttgagagtgaattaattgaacgttttggctctctagtgaagatgccattgctgaaatcggataggagtcctctgccagatcctgtgaggtcaattttggaagagggaataaatctatacgggcttcacaccaacagccatggcagaatggaatctaccaaggggtcatatgcaaaggaatgggcaaattgggagaagcggttgcgtgaagttctattcagcaatgcggagtacctcaattccattcaggttccttttgagtctgcagttaagcaagtgctggaacagctaagaaaaattgctaagggtgaatacacaacaccaattattgagaggaggaaacttggaacaattgtttttgctgctatcgatttgccagttccagaaatctgtagttccctcaacaatttggctcagaagaaccccaaggttgaagcctttcttcaggacaagcacttggagcacaaccttaagaagactcacttgacccttgcccacaagagaagtcatggcgttacagcggtagcaagttatggactgtttctcaatcagaaggtcccagtagaattgactgcacttctcttcacagataaaatggctgccctagaagcacaaccaggttctgttgatggcgaaaaagtagtttcaaaaaatgagtggccgcatattaccatatggaccgcagatggagtagcacccaaagaagccaacacactgcctcaattgttctcagaggggaaagcaactcgtgttgaattcagtccgctcatcaccatatcgggcacagtgcaattttattgagttcaattttttttttaacaaattggatttgaagcttagttttttagctgctgagaagtaatttgtataggcgaaaacaaggtg

SEQ ID NO: 21 - DNA, 4470 bp, Prunus avium
tgcccttgccctttgcagtggaagtggccttagagctttggttcatcggcgtagcggaaggtgaaaaatatgaaattatggatttttatagaaggaagagtcggcgtaggtgtgatcggagagcgggcatgaaagccgcatcgacaaccgccattgctatgcacgaagatatcttcgaggcagcccatggatatctggataaagatttgagctttactttgatcggatttctaagttcgataattcatgggcgtaaattcaaatgtctcaaatatctatgtgagcatgaacctcttcagcggcaacccctctcctccagtgaggtggggtggctgaccagaagggacagatgtcaagaaagtagataggtacgagggaggtacaggcaaaaaggaaaacaggaaaattggaatcccgagcacctctctctcccctgaacccggtcgccgcttgttcctacttccaaggtttataacacacaaaatcccagtgcagcaacctccataacccgccgtgtgtctcttccacttggctactcatccacattctctctctctctctctctctcatataaaaatacaagcgtagaaggttgcacgtcgaaagcagcgattgaatgtgggcgtcacagaaaatcatctatgctctcgctctccctcttgccttctcgtcttcgtctacagccctcgtttccggaaccttcctcttcctcaggtcctcctctccttcgtacgcatacacagccaaacctcgctttctctcgctctctttctcctcttccaattctccctcgcattcgaccatgccttacaaccagagaaggggcgggcttagagaacaaaagtggacagaaaaacaaaagactgacagccaaccaacctccacaggggattcatcagcagctgctgtggaagttgccactaacagagttggcggattgagtctcagtggaagcagtgggcagaccaatgcttcagttaaacccatacagtttgggaaggtccagtcggtaaatcagggtctagtccaaggtcagaaaggaatctggattcctaaatcatattcgacagtcagtggagctaagacaatagaagttgaagcacctgttgataaaagtacagttggaatctcaggcaatggagctggacaagcagcagataaaaaaaccagtgttggtttaagtaagttgttcaagggtgacctgttggaaaattttactgtggacaactccacatatgctcaggtgcaagtgcgcgctactttctatcccaaatttgaaaatgagaagtcagatcaggagataaggacaaggatgatagagatggtatctaatggcttggctaccttggaggtttcacttaaacactctgggtctctttttatgtacgctggtgataagggtggggcatatgccaaaaacagctttgggaatatatacactgctgtaggtgtatttgttcttggacggatgtttcgggaggcatggggacgtgaagcagcaaaaatgcaagcagagttcaatgattttcttgagaggaaccgtgtgtgcatatcaatggaactcgtaactgctgttctaggagaccacggacagcgccctaaggaagatttcgttgtagtgacagcagtcacagatttgggcaatgggaagccaaagttctatgcaacccctgagataattgctttctgtagaaaatggcgtctaccgacaaatcatgtatggctgttctcaacaaggaaagcagtgacatcactttttgctgcctttgatgctctctgcgaagaaggaactgcaacacctgtatgcatagctcttaatgaaattgcagatatatccatacctggttcaaaagagcatgtaagggagcagggtgaaatcttagagggtattgttgctcgtattgtaagccaggagagctcaaaacacatggagaaagtcctgaatgatttccctcctccaccaatggatggagttggtcttgatttgggacctagcgtaagggagctttgtgctgcaaataggtcgagtgaaaagcagcaaataaaagcgattcttgagggtgttggctcctctttttgccctgaccattcagactggcttggaactggagctggtgatgcccattccagaaatgcagataataaattggtgctatcaaaacttttacaatctcatgctgctgatttttctaccaccaaattgcaggaaatgattcgtttgatgaaagagaaacgttatcctgctgcctttaaatgttactataactaccacaaaattgattccatatcaagtgacaaccttttctataaaatggtcgtccatgtccatagtgattccgcatttcgacgttaccagaaagagatgaggtcaaagccaggattgtggcctttatatcgaggtttttttgttgacattaatttattcaaggcaagcaaggagagagctgctgagatagcaaaagacaaaagtagcattgtggaagacgttagcagtgatatgcctggaaaatatggattgggtgatgaagatgcaaacttaatgataaaattgaaatttcttacatataagctgcgaacctttttgattcgtaatggtttgtcaattctttttaaagaaggtccagctgcttataaagcctattacttgaggcaaatgaaagtatggggaacttcagcagcaaagcagagggaactcagcaagatgcttgatgaatgggctgtgtatatacgaaggaaatgtggaaacaaacagctgtcgtcatcagtgtacctcagtgaggctgagccttttcttgaacagtatgcaaaacgcagtccacaaaatcaggctctcataggatctgctggaaacttagtaaggactgaagatttcttggccattgttgagggaggaagagacgaagaaggtgatcttgagagggaccgggaggttgcaccatcaagccccagtgcctcagccagggacaccattccaaaggctgagggtctgattgtcttctttcctggactacctggttctgctaagtcagcactatgcaaggaactactaaatgccccaggtggaatgggagacgatcggccaattcaaagcctgatgggtgaccttatcaaaggaagatattggcagaaggttgctgatgagcgcaggagaaaaccatattcaataatgcttgcagacaagaatgcaccaaatgaagaagtatggagacagatagaagacatgtgccacagcaccagggcctccgcagttccagttgttcctgattctgaaggaaccgattcaaatccgttttcgcttgatgcattagcggttttcatgtttcgggtgcttcaacgtgctaatcatccgggaaaccttgacaaggaatctccaaatgctggctatgtgctgctaatgttctatcacctttatgagggcaagagtcgccgggagtttgacggcgaattagtagagcgttttggctcacttgtcaagatgccattgctgaaatctgataggaatccattgcccgatcctgtgaagtctattctggaggagggaataaatctatacaagcttcacactgccaaacatggaagagtggagtcaacaaagggaacctatgcaaaggagtgggctaaatgggagaaacagttgcgggatattttatttggcaatgcagagtatcttaattctgttcaggttccctttgagtctgctgttaaggacgtatcagaacagctgagaaaaattgcacaaggtgagtacaaaactccagatactgggaagaagaagtttggggccattgtttttgctgccgttagcttgcctgttacggaaatcagtgatctgcttgataatttggctgcgaaaaatagtgaagctggagctttccttaaagacaagcatttggagaatcttaataaggctcatgttactcttgcacataagagaagtcacggtgttactgccgtggctagttatggcaccttcctccacaaaacggtccctgtggatctaactaagctgttcttctcggataaaatggctgcacttgaagccagccttggctctgttgaaggagaaagagtagtatcgaaaaatgagtggccacatgtcaccttatggaccgcagaaggggttgcagcaaaggaggccaacaagttaccccagttgcattcagagggaaaggctacctgtattgcaattgacccacctgccaccattgatggcacgctggaatttttctgaggtttgtattcattttagaggcatgatggaccagaccaggccaggccagattgacctcgtacaatttcctttgatgatgccagtgttctatgaagagatagcttcactgctcaaatgaaggagaaaattttgtatgtcaggagaaggaaattttgacgagttgattctattgagaagttttgtgtatataggcaattgaagttttgaaatagattttgggaaaaaaaaaatttgaaata

SEQ ID NO: 22 - DNA, 4196 bp, Malus domestica
atattgtgtatcgcggaacaccgaaactcattgcgcctctcccctgaacccggtcgctgctacctagttccaaggattttacaccaaaacctcagagcagcccaggtacggacacgccgcaaactccagaagttgtctctcttccacttggcggctcatcagccacatccgcattcgttctctgggaaactctctctctctctctcatataaatatagaagcgtagtggtggcacgtccagagtagcaattatatgtgggcgtcgcagagaatcatctatgctctcgctctcgctcatcccctctcgtcttcgtcagccttcgtttccggaattttcctcttcctccggtcctcctctccttcctccgcccatcctcgctttctccctccctcgctttctctctcctcttccatctcgctcccccattccagcatgccttacaaccagcaaaggggtgggcgtacagaacaaaagtggacacaaaagcaaaagactgacagcccgtcaatgtccactggggattcttcagcagctgtcactaacagagttggtgagttgagtcttactggaagcaatgggcaggccaatgcttcagttgaacccacacagtttgggaaggtccaattggcaaatcagggtccagttcaagggcagaaaggaatttggatgcctaaatcatatgtgacagtgagcggagctaaggcggtagaagttgaagcaaatgttgatgaaagtacagttggaacccaaggaaatggagctggacaagcagcagctcaaaaaaccagagttggtttaagtaagctgttcaatggtaatctgttggaaaattttactgtggacaactccacttatgctcaggtgcaaatacgagctactttctatcccaaatttgaaaatgagaagacagatggggagattaggacaaggatgatagagatggtatctaacggcttggctaccttggaggtttcacttaaacactcagggtctctttttatgtacgccggtaataagggtggggcatatgccaaaaacagctttgggaatatatatacggctgtaggtgtatttgttcttggacggatgtttcgggaggcatggggacgtgaagcaccaaaaatgcaagaagagtttaatgatttccttgagaggaatcgtatgtgcatatcaatggaacttgtaactgctgttctaggagaccatggacaacgcccgaaagaagattttgctgtagtgacggcagtcacagatttgggcaatggaaagccaaagttctactcaacccctgagataattgctttctgtagaaaatggcgcctaccaacaaatcatgtatggctgttctcaacaaggaaatcagtgacatcattttttgctgcctttgatgcactctgcgaagaaggaactgcaacacctgtatgcatggctcttaatgaagttgcagatatatctataccaggttcaaaagatcatgtaaaggagcagggtgaaatcttagagggcattgttgctcgtattgtaagccaggaaagctcagaacatgtggaaaaagtcttgaaagatttccctcctccaccaatcgatggagctggtcttgatttgggaccgagcgcacgagatatttgtgctgcaaataggtcgagtgaaaagcagcaaatagaagcgcttcttgagggtgttggctcctctttttgccctgaccattcggactggtttggagttggagctggtgatgaccattccagaaacgcagataaatctgtgctatcaaaacttttgcaatctcatcctgcagatttttctaccaccaaattgcaggaaatgattcggttaatgaaagaaaagcgttttcctgctgcctttaaatgttaccatgactaccacaaagttgattccatatcaagtgacaaccttttctataaaatggtcatccatgtccatagtgactccgcatttaggcgttaccagaaagagatgaggtctaagccaggactgtggcctttatatcgaggtttttttgttgacattaatttattcaaggcaagcaaggagagagctgctgagatagcaaaaggcaaaagcagcattgtggaagatgggaacaatggtatgcctggaaaatatggattggctgatgaagatgcaaacttaatgataaaactgaaatttcttacatacaagctgcgaacctttttgattcgcaatggtttgtcaattctgtttaaagaaggtacagctgcttacaagacctattacgagcggcaaatgaaaatatggaatacttcagaaccaaagaagagggaactcagaaagatgcttgatgaatgggctgtgtacatacgaaggaaatgtggaaacaaaccgctttcatcatcagtttacctcagtgaggctgagccttttcttgaacagtatgcaaaacgcagtccacagaatcagtctctcattggatctgctggaaactttgtaagggctgaagatttcctggccattgttgagggaggaagagatgaagagggtgatcttgagagggagcaggaggttgcaccatcaagccccagtgcctcaggcagggacactatcccaaaggctgagggtctgattgtattctttcctggactacctggttctgctaagtcagcattatgcaaggaactacttcaagacccaggaagaatgggagatgatcgaccaattcaaagcctgatgggtgaccttatcaaaggaaaatattggcagaaggttgctgaagagcgcaagaaaaaaccatattccataatgcttgcagacaagaatgcaccaaatgaagaagtatggagacagattgaacacatgtgcaacagcactagggcctccgcggttccagtcgtgcctgattctgaaggaaccgattcaaatccattttctcttgatgcattagcaattttcatgtttcgggtgcttcaacgtgctaatcatccaggaaaccttgacaaggaatctttaaatgctggctatgtgctgctaatgttctatcacctttacgagggcaagagtcgccgagagtttgatggggaattagttgagcgttttggctcacttgtaaagatgccgttgctgaagtctgataggaatccattacctgatcccgtgaagaatattctggaggagggaataaatctatacaagcttcacaccgccaaacatggaagattggagtcgaccaagggaacctatgcaaaggagtgggctaaatgggagaaacagttgcgggatattttatttggcaatgctgagtatctgaattctgttcaggttccttttgagtctgctgtaaaggaagtgtcagaacagctgaaaaaggtcgcaaaaggtgagtacaaaactccagatactgggaagaggaagttcggcgccattgtctttgctgccgttagcctgcctgttatggaagtcagtggtctgcttgatagcttggctgtgaaacatagtgaagccgaagctttcctcaaagacaagcatttggataaacttaacaaggctcatgttactcttgcacacaagagaagtcatggtgttactgccgtggctagttacggaaccttccttcacaaaacggtccctgtggatataactaagcttttcttctcggataaaatggctgcatttggagccagccttgggtctgtcgaaggtgaaagagtagtgtctaaaaatgagtggccgcatgtcaccttatggactgcagaaggggttccggccaaggacgccaacaacttaccccaattgcattcggaggggaaagctacctgcattgcaattgacccacctgccaccattgatggcacgctggaatttttctgaggtttgatcggccaggccagattgagctcggcatacgattggagtgaaatttcatttgacgatgcgggtgttcaatgaagagagaacttaactgcttaagtgaaggagaaaattttgtaagccatgaggaaaaggaaattttgttgagttgatttcttttcagaggttttgtatacataaggcaattaaaattttaaagtctcagcgttgcttcatcagcttttaccaattgaggggtgtttagccgcggtcgcatcgctcgtatctgtttacacgattcggtatgattgcgcagctgcaactcccccaagttttatgacacttgaaatgttgacactgcattttttta

SEQ ID NO: 23 - DNA, 517 bp, Tetrahymena termophila
tgacgcaattcaaccaagcgcgggtaaacggcgggagtaactatgactctctaaatagcaatatttacctttggagggaaaagttatcaggcatgcacctggtagctagtctttaaaccaatagattgcatcggtttaaaaggcaagaccgtcaaattgcgggaaaggggtcaacagccgttcagtaccaagtctcaggggaaactttgagatggccttgcaaagggtatggtaataagctgacggacatggtcctaaccacgcagccaagtcctaagtcaacagatcttctgttgatatggatgcagttcacagactaaatgtcggtcggggaagatgtattcttctcataagatatagtcggacctctccttaatgggagctagcggatgaagtgatgcaacactggagccgctgggaactaatttgtatgcgaaagtatattgattagttttggagtactcgtaaggtagccaaatgcctcgtcatctaattagtgacgcgcatgaatggatta

SEQ ID NO: 24 - DNA, 174 bp, Ceratitis capitata
gatgacatggagaagatctggcaccacaccttctacaacgagttgcgtgtcgcccccgaggagcaccccgttctgctgaccgaagcaccgttgaacccgaaggctaaccgcgagaagatgacccagatcatgttcgagaccttcaactcgccggccatgtatgtggccatccag